European Patent Application EP 4 461 740 A1, published November 13, 2024. Title: A MODIFIED YEAST STRAIN FOR LOW ALCOHOL FERMENTATION. Applicant: BRAIN Biotech AG. The sequence listing filed with the application follows.

SEQUENCE LISTING (9 sequences)

SEQ ID NO: 1 - protein, 240 aa, unidentified
MADEERLKEFKEANKIVFDPNTRQVWENQNRDGTKPATTFQSEEDMKRAAPESEKGTSATSGIVPTLQNIVATVTLGCRLDLKTVALHARNAEYNPKRFAAVIMRIREPKTTALIFAPGKMVVTGAKSEDDSKLASRKYARIIQKIGFAAKFTDFKIQNIVGSCDVKFPIRLEGLAFSHGTFSSYEPELFPGLIHRMVKPKIVLSIFVSGKIVLTGAKQREEIYQAFEAIYPVLSEFRKM

SEQ ID NO: 2 - DNA, 723 bp, unidentified
  source 1..723: mol_type = other DNA
atggccgatgaggaacgtttaaaggagtttaaagaggcaaacaagatagtgtttgatccaaataccagacaagtatgggaaaaccagaatcgagatggtacaaaaccagcaactactttccagagtgaagaggacatgaaaagagctgccccagaatctgaaaaaggtacctccgccacatcaggtattgttccaacactacaaaacattgtggcaactgtgactttggggtgcaggttagatctgaaaacagttgcgctacatgcccgtaatgcagaatataaccccaagcgttttgctgctgtcatcatgcgtattagagagccaaaaactacagctttaatttttgccccagggaaaatggttgttaccggtgcaaaaagtgaggatgactcaaagctggccagtagaaaatatgcaagaattatccaaaaaatcgggtttgctgctaaattcacagacttcaaaatacaaaatattgtcggttcgtgtgacgttaaattccctatacgtctagaagggttagcattcagtcatggtactttctcctcctatgagccagaattgtttcctggtttgatccatagaatggtgaagccgaaaattgtgttgagtatttttgtttcaggaaagattgttcttactggtgcaaagcaaagggaagaaatttaccaagcttttgaagctatataccctgtgctaagtgaatttagaaaaatgtga

SEQ ID NO: 3 - DNA, 3822 bp, unidentified
  source 1..3822: mol_type = other DNA
atgaagaacagcctggaagatttcaccaacctgtacagcctgcagaaaaccctgagattcgagctgaagcccatcggcaacacccagagcatgctggaagaggacggcgtgttcgacaccgacgagaagagaaagatcgcctacagcaagaccaagccttacatcgaccggctgcacagagagttcatcgaggaaagcctgagcgacgcccagatcagcaagctggacgagtacttcaaggcctacgtggactacaagaaggataagaaggacaccaagcggttcaaccggatcaagcagttcaagagcgtgctgcggaaagaagtggtggatcacttcaacaagcagggcaaagaatggaccaccgtgaagttcgcccacctgaagatcaagaaaaaggacctggaagtgctgttcgagaagcagctgcccaacatcctgaaagaggaatacggcaccgagaaagagacacagatcatcgacgaggacagcggcgaagtgaccagcatcttcgacatgtggaacggcttcatgggctacttcaccaagttcttcgagacacggaagaacttctacaagagcgacggcaccagcaccgccattgccaccagaatcatcgaccagaacctggacagattcatcgagaacatcctcatctacgacagcatcaagcccaagatcgacaccagcgaagtgcgcgagttcttcaacctggaaagcgacaccatcttcagcatggaattctacaacaactgcctgctgcaggccggcatcgatcagtacaacaatttcctcggcggcaagaccctggaaaacggcagaaagatccggggcatcaacgagctgatcaacaagtaccggcaagagaaccccgaggacaagatcccattcctgaagaagctggacaagcagatccacagcgagaaagaaaagttcatccagcagatcgagacactcgaggacctgaaagaagaactgcagaagttctacaactccagcaacgagaagattaagatcctggacaacctgctgtcccggatcgaggaattcaagcccgagggcatcttcatctccaagcaggccttcaacaccatcagcagacggtggaccgatcagagcgaggcctttgagacaagcctgttcgagtccctcaaagaggaaaagcccatcaccggcacagccaaaaagaaggatgacggctacaacttccccgagttcatctccctgcagagcatccggaacacactgaagaaggtgcagggcgaagagaggttctggaaagagcggtactaccgggacaacagcgagtctggaatcctggccggcaacgaggaaatctggacccagttcctgatgatcttcaagtccgagttcaacagcaagttcgagcggaacgaccctgaggacaatggcaccatcggctacaatctgtttaaagaggacctcgagaagctgctcaaggacctcaagatcaccaaggataccaagagcatcatcaagcgcttcgccgacgaggccctgcacatctatcaagtgggcaagtatttcgccctcgagaaagacagagtgtggatcagcagctacgacgacctgctggacaccttctacacagaccccaacaccggctacctgagcttttacgagggcgcctacgagcagatcgtgcagccctacaacatgatccggaactacctgaccagaaagccctactccgatgagaagtggaagctgaacttcgagaaccccacactggccaacggctgggacaagaacaaagagacagacaacagctccatcatgctgagaaaagaaggcgcctactacctgggcatcatgaagaagggcaagaacaagctgtttgaggaacggaaccggcagctgttcgaacccaagaacggcgaggatacctacgagaaactgagctataagctgttccccgatcctgccaagatgatccccaaagtgtgcttcagcaacaagaacatccagatgttcagccccagcaccgagatcatgaacatctacaacggcgagacattcaagaagaatagcgacgacttcagcgtgtcctccatgcagaagctgatcgccttttacaccaagtgcctgagccagtacgaaggctggaagtactacgacttcaagtacatcaagagccccgaccagtacaaggacaacatcggcgagttttacaacgacgtggccaagagcggctacagagtttggttcgagaatatcagccagagctacgtcgacagcaagaacaccatgggcgagctgtacctgttcaagatccacaacaaggactggaaccagaaggacaaaaagaccaaagtgggctccaagaacctgcacacccactacttcgaggaactgttcagccaggacaatattgagaacaactttccgctgaagctgaatggcgaggccgaggtgttctacagacccaagacaaacccagagaagctgggcaccaagaaggactctaagggcagagaagtgatcgaccggaagagatacgccagcgacaaggtgctgttccacgtgccaatcacactgaacagaacccctgtgaccaccaccaagctgaacaaagaaatcaacggcttcctggccaacaatcccagcatcaacatcatcggcgtggaccggggagagaagcacctggtgtactacagcgtggtcaaccagcggggcaaaatgctggaatccggctcctttaataccatcaacggcgtcgactaccacggcaaactggaagagagagccgatcggagagagcaggctagaagagactggcaggacgtggaaggcatcaagaatctgaagaaaggctacatcagcctggtcgtcagagagctggccaacctgagcatcaagtacaacgccatcatcgtgatggaagatctgaacatgcggtttaagcagatcagaggcggcatcgagaagtccgcctaccagcagctggaaaaggccctgatcgaaaagctgaattacctggtcaacaagaccgagacagaccctcagaaaaccggccacattctgaaggcctatcagctgacaagccccatcaagtcctttaaagagatgggcaagcagaccggcatcatcttctacacccaagccagctacaccagcgtgaccgatcctatcacaggctggcggcccaatctgtacctgaagtacagcagcgccagcaaggccaagtccgatatcctgaagttctccaagatctcctacaacaccaacaacaaccgcttcgagttcacctacgacctgcggaacttcgtgaacatgaaggcttatccccagaaaactgcctggaccatctgcagcaacgtggaaagattccgctgggacagaaagggcaacaaaaacaacggggagtacatccagtataaggacctgaccgagaatttcaagaccttctttgaggaagtgtccatcaactacaaaggcgacatcctgttccagatcaaaaacctgagcgagaaggggaacgagaagtttttccgggacctgatcttctatatcagcctgatctcccagatacggaacacccaaaaggacaagaagggcgacgagaacgacttcattctgagccccgtggaaccattcttcgacagcagaaagagcagcaccttcggcgagaatctgcccctgaacggggatgccaatggcgcctacaatatcgcccggaagggcatcattatgctgaacaagattagcaagggctccaaaaacaaagtcaaagaagatatcggctggggcgacctgtacatccctcacaccgagtgggatgatttcgccaccggctccatt

SEQ ID NO: 4 - DNA, 23 bp, unidentified
  source 1..23: mol_type = other DNA
gaactggaatatctttgtattcc

SEQ ID NO: 5 - DNA, 8235 bp, unidentified
  source 1..8235: mol_type = other DNA
agcttgcaaattaaagccttcgagcgtcccaaaaccttctcaagcaaggttttcagtataatgttacatgcgtacacgcgtctgtacagaaaaaaaagaaaaatttgaaatataaataacgttcttaatactaacataactataaaaaaataaatagggacctagacttcaggttgtctaactccttccttttcggttagagcggatgtggggggagggcgtgaatgtaagcgtgacataactaattacatgatatcgacaaaggaaaagggggacggatctccgaggcctcggacccgtcgggccgcgtcggacgtgtcagtcctgctcctcgcaattgttagaaaaactcatcgagcatcaaatgaaactgcaatttattcatatcaggattatcaataccatatttttgaaaaagccgtttctgtaatgaaggagaaaactcaccgaggcagttccataggatggcaagatcctggtatcggtctgcgattccgactcgtccaacatcaatacaacctattaatttcccctcgtcaaaaataaggttatcaagtgagaaatcaccatgagtgacgactgaatccggtgagaatggcaaaagcttatgcatttctttccagacttgttcaacaggccagccattacgctcgtcatcaaaatcactcgcatcaaccaaaccgttattcattcgtgattgcgcctgagcgaggcgaaatacgcgatcgctgttaaaaggacaattacaaacaggaatcgaatgcaaccggcgcaggaacactgccagcgcatcaacaatattttcacctgaatcaggatattcttctaatacctggaatgctgttttgccggggatcgcagtggtgagtaaccatgcatcatcaggagtacggataaaatgcttgatggtcggaagaggcataaattccgtcagccagtttagtctgaccatctcatctgtaacatcattggcaacgctacctttgccatgtttcagaaacaactctggcgcatcgggcttcccatacaatcgatagattgtcgcacctgattgcccgacattatcgcgagcccatttatacccatataaatcagcatccatgttggaatttaatcgcggcctcgaaacgtgagtcttttccttacccatggtttagttcctcaccttgtcgtattatactatgccgatatactatgccgatgattaattgtcaacaccgcccttagattagattgctatgctttctttctaatgagcaagaagtaaaaaaagttgtaatagaacaagaaaaatgaaactgaaacttgagaaattgaagaccgtttattaacttaaatatcaatgggaggtcatcgaaagagaaaaaaatcaaaaaaaaaaattttcaagaaaaagaaacgtgataaaaatttttattgcctttttcgacgaagaaaaagaaacgaggcggtctcttttttcttttccaaacctttagtacgggtaattaacgacaccctagaggaagaaagaggggaaatttagtatgctgtgcttgggtgttttgaagtggtacggcgatgcgcggagtccgagaaaatctggaagagtaaaaaaggagtagaaacattttgaagctatggtgtgtgggggatccgcacaaacgaaggtctcactgatcgcttgcctgtaacttacacgcgcctcgtatcttttaatgatggaataatttgggaatttactctgtgtttatttatttttatgttttgtatttggattttagaaagtaaataaagaaggtagaagagttacggaatgaagaaaaaaaaataaacaaaggtttaaaaaatttcaacaaaaagcgtactttacatatatatttattagacaagaaaagcagattaaatagatatacattcgattaacgataagtaaaatgtaaaatcacaggattttcgtgtgtggtcttctacacagacaagatgaaacaattcggcattaatacctgagagcaggaagagcaagataaaaggtagtatttgttggcgatccccctagagtcttttacatcttcggaaaacaaaaactattttttctttaatttctttttttactttctatttttaatttatatatttatattaaaaaatttaaattataattatttttatagcacgtgatgaaaaggacccatcgataagctggtacgcgccatatggcctgcaggtttaaagattacggatatttaacttacttagaataatgccatttttttgagttataataatcctacgttagtgtgagcgggatttaaactgtgaggaccttaatacattcagacacttctgcggtatcaccctacttattcccttcgagattatatctaggaacccatcaggttggtggaagattacccgttctaagacttttcagcttcctctattgatgttacacctggacaccccttttctggcatccagtttttaatcttcagtggcatgtgagattctccgaaattaattaaagcaatcacacaatgctctcggataccacctcggttgaaactgacaggtggtttgttacgcatgctaatgcaaaggagcctatatacctttggctcggctgctgtaacagggaatataaagggcagcataatttaggagtttagtgaacttgcaacatttactattttcccttcttacgtaaatatttttctttttaattctaaatcaatctttttcaattttttgtttgtattcttttcttgcttaaatctataactacaaaaaacacatacataaactaaaaatggccgactacaaggacgacgacgataagggcgctgccgagaacctgtactttcagtctcctgccgccaagaagaagaaactggacggcagcgtggacatgaagaacagcctggaagatttcaccaacctgtacagcctgcagaaaaccctgagattcgagctgaagcccatcggcaacacccagagcatgctggaagaggacggcgtgttcgacaccgacgagaagagaaagatcgcctacagcaagaccaagccttacatcgaccggctgcacagagagttcatcgaggaaagcctgagcgacgcccagatcagcaagctggacgagtacttcaaggcctacgtggactacaagaaggataagaaggacaccaagcggttcaaccggatcaagcagttcaagagcgtgctgcggaaagaagtggtggatcacttcaacaagcagggcaaagaatggaccaccgtgaagttcgcccacctgaagatcaagaaaaaggacctggaagtgctgttcgagaagcagctgcccaacatcctgaaagaggaatacggcaccgagaaagagacacagatcatcgacgaggacagcggcgaagtgaccagcatcttcgacatgtggaacggcttcatgggctacttcaccaagttcttcgagacacggaagaacttctacaagagcgacggcaccagcaccgccattgccaccagaatcatcgaccagaacctggacagattcatcgagaacatcctcatctacgacagcatcaagcccaagatcgacaccagcgaagtgcgcgagttcttcaacctggaaagcgacaccatcttcagcatggaattctacaacaactgcctgctgcaggccggcatcgatcagtacaacaatttcctcggcggcaagaccctggaaaacggcagaaagatccggggcatcaacgagctgatcaacaagtaccggcaagagaaccccgaggacaagatcccattcctgaagaagctggacaagcagatccacagcgagaaagaaaagttcatccagcagatcgagacactcgaggacctgaaagaagaactgcagaagttctacaactccagcaacgagaagattaagatcctggacaacctgctgtcccggatcgaggaattcaagcccgagggcatcttcatctccaagcaggccttcaacaccatcagcagacggtggaccgatcagagcgaggcctttgagacaagcctgttcgagtccctcaaagaggaaaagcccatcaccggcacagccaaaaagaaggatgacggctacaacttccccgagttcatctccctgcagagcatccggaacacactgaagaaggtgcagggcgaagagaggttctggaaagagcggtactaccgggacaacagcgagtctggaatcctggccggcaacgaggaaatctggacccagttcctgatgatcttcaagtccgagttcaacagcaagttcgagcggaacgaccctgaggacaatggcaccatcggctacaatctgtttaaagaggacctcgagaagctgctcaaggacctcaagatcaccaaggataccaagagcatcatcaagcgcttcgccgacgaggccctgcacatctatcaagtgggcaagtatttcgccctcgagaaagacagagtgtggatcagcagctacgacgacctgctggacaccttctacacagaccccaacaccggctacctgagcttttacgagggcgcctacgagcagatcgtgcagccctacaacatgatccggaactacctgaccagaaagccctactccgatgagaagtggaagctgaacttcgagaaccccacactggccaacggctgggacaagaacaaagagacagacaacagctccatcatgctgagaaaagaaggcgcctactacctgggcatcatgaagaagggcaagaacaagctgtttgaggaacggaaccggcagctgttcgaacccaagaacggcgaggatacctacgagaaactgagctataagctgttccccgatcctgccaagatgatccccaaagtgtgcttcagcaacaagaacatccagatgttcagccccagcaccgagatcatgaacatctacaacggcgagacattcaagaagaatagcgacgacttcagcgtgtcctccatgcagaagctgatcgccttttacaccaagtgcctgagccagtacgaaggctggaagtactacgacttcaagtacatcaagagccccgaccagtacaaggacaacatcggcgagttttacaacgacgtggccaagagcggctacagagtttggttcgagaatatcagccagagctacgtcgacagcaagaacaccatgggcgagctgtacctgttcaagatccacaacaaggactggaaccagaaggacaaaaagaccaaagtgggctccaagaacctgcacacccactacttcgaggaactgttcagccaggacaatattgagaacaactttccgctgaagctgaatggcgaggccgaggtgttctacagacccaagacaaacccagagaagctgggcaccaagaaggactctaagggcagagaagtgatcgaccggaagagatacgccagcgacaaggtgctgttccacgtgccaatcacactgaacagaacccctgtgaccaccaccaagctgaacaaagaaatcaacggcttcctggccaacaatcccagcatcaacatcatcggcgtggaccggggagagaagcacctggtgtactacagcgtggtcaaccagcggggcaaaatgctggaatccggctcctttaataccatcaacggcgtcgactaccacggcaaactggaagagagagccgatcggagagagcaggctagaagagactggcaggacgtggaaggcatcaagaatctgaagaaaggctacatcagcctggtcgtcagagagctggccaacctgagcatcaagtacaacgccatcatcgtgatggaagatctgaacatgcggtttaagcagatcagaggcggcatcgagaagtccgcctaccagcagctggaaaaggccctgatcgaaaagctgaattacctggtcaacaagaccgagacagaccctcagaaaaccggccacattctgaaggcctatcagctgacaagccccatcaagtcctttaaagagatgggcaagcagaccggcatcatcttctacacccaagccagctacaccagcgtgaccgatcctatcacaggctggcggcccaatctgtacctgaagtacagcagcgccagcaaggccaagtccgatatcctgaagttctccaagatctcctacaacaccaacaacaaccgcttcgagttcacctacgacctgcggaacttcgtgaacatgaaggcttatccccagaaaactgcctggaccatctgcagcaacgtggaaagattccgctgggacagaaagggcaacaaaaacaacggggagtacatccagtataaggacctgaccgagaatttcaagaccttctttgaggaagtgtccatcaactacaaaggcgacatcctgttccagatcaaaaacctgagcgagaaggggaacgagaagtttttccgggacctgatcttctatatcagcctgatctcccagatacggaacacccaaaaggacaagaagggcgacgagaacgacttcattctgagccccgtggaaccattcttcgacagcagaaagagcagcaccttcggcgagaatctgcccctgaacggggatgccaatggcgcctacaatatcgcccggaagggcatcattatgctgaacaagattagcaagggctccaaaaacaaagtcaaagaagatatcggctggggcgacctgtacatccctcacaccgagtgggatgatttcgccaccggctccattaagaggccagccgccacaaagaaagccggacaggctaaaaagaagaaggccagcggaagcggcgctggcagcccgaaaaagaaacgcaaggtggaagatcccaagaagaaacggaaagtctgagcggccgcaatgccggcgcaatgattgaatagtcaaagattttttttttttaattttttttttttaattttttttttttttcatagaactttttatttaaataaatcacgtctatatatgtatcagtataacgtaaaaaaaaaaacaccgtcagttaaacaaaacataaataaaaaaaaaaagaagtgtcaaatcaagtgtcaaatggccctgcattaatgaatcggccaacgcgcggggagaggcggtttgcgtattgggcgctcttccgcttcctcgctcactgactcgctgcgctcggtcgttcggctgcggcgagcggtatcagctcactcaaaggcggtaatacggttatccacagaatcaggggataacgcaggaaagaacatgtgagcaaaaggccagcaaaaggccaggaaccgtaaaaaggccgcgttgctggcgtttttccataggctccgcccccctgacgagcatcacaaaaatcgacgctcaagtcagaggtggcgaaacccgacaggactataaagataccaggcgtttccccctggaagctccctcgtgcgctctcctgttccgaccctgccgcttaccggatacctgtccgcctttctcccttcgggaagcgtggcgctttctcatagctcacgctgtaggtatctcagttcggtgtaggtcgttcgctccaagctgggctgtgtgcacgaaccccccgttcagcccgaccgctgcgccttatccggtaactatcgtcttgagtccaacccggtaagacacgacttatcgccactggcagcagccactggtaacaggattagcagagcgaggtatgtaggcggtgctacagagttcttgaagtggtggcctaactacggctacactagaagaacagtatttggtatctgcgctctgctgaagccagttaccttcggaaaaagagttggtagctcttgatccggcaaacaaaccaccgctggtagcggtggtttttttgtttgcaagcagcagattacgcgcagaaaaaaaggatctcaagaagatcctttgatcttttctacggggtctgacgctcagtggaacgaaaactcacgttaagggattttggtcatgagattatcaaaaaggatcttcacctagatccttttaaattaaaaatgaagttttaaatcaatctaaagtatatatgagtaaacttggtctgacagttaccaatgcttaatcagtgaggcacctatctcagcgatctgtctatttcgttcatccatagttgcctgactccccgtcgtgtagataactacgatacgggagggcttaccatctggccccagtgctgcaatgataccgcgagacccacgctcaccggctccagatttatcagcaataaaccagccagccggaagggc

SEQ ID NO: 6 - DNA, 6488 bp, unidentified
  source 1..6488: mol_type = other DNA
ccccgtagaaaagatcaaaggatcttcttgagatcctttttttctgcgcgtaatctgctgcttgcaaacaaaaaaaccaccgctaccagcggtggtttgtttgccggatcaagagctaccaactctttttccgaaggtaactggcttcagcagagcgcagataccaaatactgtccttctagtgtagccgtagttaggccaccacttcaagaactctgtagcaccgcctacatacctcgctctgctaatcctgttaccagtggctgctgccagtggcgataagtcgtgtcttaccgggttggactcaagacgatagttaccggataaggcgcagcggtcgggctgaacggggggttcgtgcacacagcccagcttggagcgaacgacctacaccgaactgagatacctacagcgtgagctatgagaaagcgccacgcttcccgaagggagaaaggcggacaggtatccggtaagcggcagggtcggaacaggagagcgcacgagggagcttccagggggaaacgcctggtatctttatagtcctgtcgggtttcgccacctctgacttgagcgtcgatttttgtgatgctcgtcaggggggcggagcctatggaaaaacgccagcaacgcggcctttttacggttcctgggcttttgctggccttttgctcacatgttctttcctgcgttatcccctgattctgtggataaccgtattaccgcctttgagtgagctgataccgctcgccgcagccgaacgaccgagcgcagcgagtcagtgagcgaggaagcggaagagcgcccaatacgcaaaccgcctctccccgcgcgttggccgattcattaatgcagggccgcagcttgcaaattaaagccttcgagcgtcccaaaaccttctcaagcaaggttttcagtataatgttacatgcgtacacgcgtctgtacagaaaaaaaagaaaaatttgaaatataaataacgttcttaatactaacataactataaaaaaataaatagggacctagacttcaggttgtctaactccttccttttcggttagagcggatgtggggggagggcgtgaatgtaagcgtgacataactaattacatgatgcggccctctagatgcatgctcgaggagctcggatcccggtctgcatctgcggatcctctttgaaaagataatgtatgattatgctttcactcatatttatacagaaacttgatgttttctttcgagtatatacaaggtgattacatgtacgtttgaagtacaactctagattttgtagtgccctcttgggctagcggtaaaggtgcgcattttttcacaccctacaatgttctgttcaaaagattttggtcaaacgctgtagaagtgaaagttggtgcgcatgtttcggcgttcgaaacttctccgcagtgaaagataaatgatctagttttcacaagaaaacaagcgcaagtggtttagtggtaaaatccaacgttgccatcgttgggcccccggttcgattccgggcttgcgcaaatttctactgttgtagatgaactggaatatctttgtattccatttattttttgtcactattgttatgtaaaatgccacctctgacagtatggaacgcaaacttctgtctagtggataacagaatttttctatggccaatttaaccggtgaggacgaggacgcacggaggagagtcttccttcggagggctgtcacccgctcggcggcttctaatccgtggactagtggatcgatccccacgcgccctgtagcggcgcattaagcgcggcgggtgtggtggttacgcgcagcgtgaccgctacacttcccaccgccctagcccccgctcctttcgctttcttcccttcctttctcgccacgttcgccggctttccccgtcaagctctaaatgggggcatccgtttacccttccgatttactgctttacggcacctcgaccccaaaaaacttgattagggtgatggttcacgtagtgggccatcgccctgatagaccctttttcgccctttgacgttggagtccacgttctttaatagtggactcttgttggaaactggaacaacactcaaccctatctcggtctattcttttgatttataagggattttgccgatttcgggctattcgttaaaaaatgagctgatttaacaaaaatttaacgcgaattttaacaaaatattaacgtttacaatttaaatatttgcttatacaatcttcctgtttttggggcttttctgattatcaaccggggtggagcttcccattgcgaataccgcttccacaaacattgctcaaaagtatctctttgctatatatctctgtgctatatccctatataacctacccatccacctttcgctccttgaacttgcatctaaactcgacctctacattttttatgtttatctctagtattactctttagacaaaaaaattgtagtaagaactattcatagagtgaatcgaaaacaatacgaaaatgtaaacatttcctatacgtagtatatagagacaaaatagaagaaaccgttcataattttctgaccaatgaagaatcatcaacgctatcactttctgttcacaaagtatgcgcaatccacatcggtatagaatataatcggggatgcctttatcttgaaaaaatgcacccgcagcttcgctagtaatcagtaaacgcgggaagtggagtcaggctttttttatggaagagaaaatagacaccaaagtagccttcttctaaccttaacggacctacagtgcaaaaagttatcaagagactgcattatagagcgcacaaaggagaaaaaaagtaatctaagatgctttgttagaaaaatagcgctctcgggatgcatttttgtagaacaaaaaagaagtatagattctttgttggtaaaatagcgctctcgcgttgcatttctgttctgtaaaaatgcagctcagattctttgtttgaaaaattagcgctctcgtcgcgttgcatttttgttttacaaaaatgaagcacagattcttcgttggtaaaatagcgctttcgcgttgcatttctgttctgtaaaaatgcagctcagattctttgtttgaaaaattagcgctctcgcgttgcatttttgttctacaaaatgaagcacagatgcttcgttaacaaagatatgctattgaagtgcaagatggaaacgcagaaaatgaaccggggatgcgacgtgcaagattacctatgcaatagatgcaatagtttctccaggaaccgaaatacatacattgtcttccgtaaagcgctagactatatattattatacaggttcaaatatactatctgtttcagggaaaactcccaggttcggatgttcaaaattcaatgatgggtaacaagtacgatcgtaaatctgtaaaacagtttgtcggatattaggctgtatctcctcaaagcgtattcgaatatcattgagaagctgcagcgtcacatcggataataatgatggcagccattgtagaagtgccttttgcatttctagtctctttctcggtctagctagttttactacatcgcgaagatagaatcttagatcacactgcctttgctgagctggatcaatagagtaacaaaagagtggtaaggcctcgttaaaggacaaggacctgagcggaagtgtatcgtacagtagacggagtatctagtatagtctatagtccgtggaattaattctcatctttgacagcttatcatcgataagtttagcttgcctcgtccccgccgggtcacccggccagcgacatggaggcccagaataccctccttgacagtcttgacgtgcgcagctcaggggcatgatgtgactgtcgcccgtacatttagcccatacatccccatgtataatcatttgcatccatacattttgatggccgcacggcgcgaagcaaaaattacggctcctcgctgcagacctgcgagcagggaaacgctcccctcacagacgcgttgaattgtccccacgccgcgcccctgtagagaaatataaaaggttaggatttgccactgaggttcttctttcatatacttccttttaaatcttgctaggatacagttctcacatcacatccgaacataaacaaccatgggtaaaaagcctgaactcaccgcgacgtctgtcgagaagtttctgatcgaaaagttcgacagcgtctccgacctgatgcagctctcggagggcgaagaatctcgtgctttcagcttcgatgtaggagggcgtggatatgtcctgcgggtaaatagctgcgccgatggtttctacaaagatcgttatgtttatcggcactttgcatcggccgcgctcccgattccggaagtgcttgacattggggaatttagcgagagcctgacctattgcatctcccgccgtgcacagggtgtcacgttgcaagacctgcctgaaaccgaactgcccgctgttctgcagccggtcgcggaggcaatggatgcgatcgctgcggccgatcttagccagacgagcgggttcggcccattcggaccgcaaggaatcggtcaatacactacatggcgtgatttcatatgcgcgattgctgatccccatgtgtatcactggcaaactgtgatggacgacaccgtcagtgcgtccgtcgcgcaggctctcgatgagctgatgctttgggccgaggactgccccgaagtccggcacctcgtgcacgcggatttcggctccaacaatgtcctgacggacaatggccgcataacagcggtcattgactggagcgaggcgatgttcggggattcccaatacgaggtcgccaacatcttcttctggaggccgtggttggcttgtatggagcagcagacgcgctacttcgagcggaggcatccggagcttgcaggatcgccgcggctccgggcgtatatgctccgcattggtcttgaccaactctatcagagcttggttgacggcaatttcgatgatgcagcttgggcgcagggtcgatgcgacgcaatcgtccgatccggagccgggactgtcgggcgtacacaaatcgcccgcagaagcgcggccgtctggaccgatggctgtgtagaagtactcgccgatagtggaaaccgacgccccagcactcgtccgagggcaaaggaataatcagtactgacaataaaaagattcttgttttcaagaacttgtcatttgtatagtttttttatattgtagttgttctattttaatcaaatgttagcgtgatttatattttttttcgcctcgacatcatctgcccagatgcgaagttaagtgcgcagaaagtaatatcatgcgtcaatcgtatgtgaatgctggtcgctatactgctgtcgattcgatactaacgccgccatccagtgtcgaaaatactaaactcacaaattagagcttcaatttaattatatcagttattacccattgaaaaaggaagagtatgagtattcaacatttccgtgtcgcccttattcccttttttgcggcattttgccttcctgtttttgctcacccagaaacgctggtgaaagtaaaagatgctgaagatcagttgggtgcacgagtgggttacatcgaactggatctcaacagcggtaagatccttgagagttttcgccccgaagaacgttttccaatgatgagcacttttaaagttctgctatgtgatacactattatcccgtattgacgccgggcaagagcaactcggtcgccgcatacactattctcagaatgacttggttgagtactcaccagtcacagaaaagcatcttacggatggcatgacagtaagagaattatgcagtgctgccataaccatgagtgataacactgcggccaacttacttctgacaacgatcggaggaccgaaggagctaaccgcttttttgcacaacatgggggatcatgtaactcgccttgatcgttgggaaccggagctgaatgaagccataccaaacgacgagagtgacaccacgatgcctgtagcaatgccaacaacgttgcgcaaactattaactggcgaactacttactctagcttcccggcaacaattaatagactgaatggaggcggataaagttgcaggaccacttctgcgctcggcccttccggctggctggtttattgctgataaatctggagccggtgagcgtgggtctcgcggtatcattgcagcactggggccagatggtaagcgctcccgtatcgtagttatctacacgacggggagtcaggcaactatggatgaacgaaatagacagatcgctgagataggtgcctcactgattaagcattggtaactgtcagaccaagtttactcatatatactttagattgatttaaaacttcatttttaatttaaaaggatctaggtgaagatcctttttgataatctcatgaccaaaatcccttaacgtgagttttcgttccactgagcgtcaga

SEQ ID NO: 7 - DNA, 1760 bp, unidentified
  source 1..1760: mol_type = other DNA
gttgttgtctcaccatatccgcaatgacaaaaaaatgatggaagacactaaaggaaaaaattaacgacaaagacagcaccaacagatgtcgttgttccagagctgatgaggggtatctcgaagcacacgaaactttttccttccttcattcacgcacactactctctaatgagcaacggtatacggccttccttccagttacttgaatttgaaataaaaaaagtttgctgtcttgctatcaagtataaatagaactgcaattattaatcttttgttttctcgtcattgttctcgttccctttcttccttgtttctttttctgcacaatatttcaagctataccaagcatacaatcaactatctcatatacaatggccgatgaggaacgtttaaaggagtttaaagaggcaaacaagatagtgtttgatccaaataccagacaagtatgggaaaaccagaatcgagatggtacaaaaccagcaactactttccagagtgaagaggacatgaaaagagctgccccagaatctgaaaaaggtacctccgccacatcaggtattgttccaacactacaaaacattgtggcaactgtgactttggggtgcaggttagatctgaaaacagttgcgctacatgcccgtaatgcagaatataaccccaagcgttttgctgctgtcatcatgcgtattagagagccaaaaactacagctttaatttttgccccagggaaaatggttgttaccggtgcaaaaagtgaggatgactcaaagctggccagtagaaaatatgcaagaattatccaaaaaatcgggtttgctgctaaattcacagacttcaaaatacaaaatattgtcggttcgtgtgacgttaaattccctatacgtctagaagggttagcattcagtcatggtactttctcctcctatgagccagaattgtttcctggtttgatccatagaatggtgaagccgaaaattgtgttgagtatttttgtttcaggaaagattgttcttactggtgcaaagcaaagggaagaaatttaccaagcttttgaagctatataccctgtgctaagtgaatttagaaaaatgtgatggggaaggagtagacgaaaagaaaaaaaggttttctatttgttccattttctcaattattaatggtcctcaaagaaataaaagaaaaggaagaagaagtaattgtaatatcaaacggttttttatagtatattcttcttattctatatttatatatcaatgttttataataagatgtttattcatagcatatctggtggatcgtctctattaagcgccagcgaggtgtttgcctctgcatttttcagcaaagcaagctccctttccagcttgaatctatgttcacgctcatccgacaacgaatttcttatgatttatgatttttattattaaataagttataaaaaaataagtgtatacaaattttaaagtgactcttaggttttaaaacgaaaattcttattcttgagtaactctttcctgtaggtcaggttgctttctcaggtatagcatgaggtcgctcttattgaccacatctctaccggcatgccgagcaaatgcctgcaaatcgctccccatttcacccaattgtagatatgctaactccagcaatgagttgatgaatctcggtgtgtattttatgtcctcagaggacaacacctgttgtaatcgttcttccacacggatccacagcctagccttcagttgggctctatcttcatcgtc

SEQ ID NO: 8 - DNA, 723 bp, Saccharomyces cerevisiae
  source 1..723: mol_type = other DNA
atggccgatgaggaacgtttaaaggagtttaaagaggcaaacaagatagtgtttgatccaaataccagacaagtatgggaaaaccagaatcgagatggtacaaaaccagcaactactttccagagtgaagaggacataaaaagagctgccccagaatctgaaaaagacacctccgccacatcaggtattgttccaacactacaaaacattgtggcaactgtgactttggggtgcaggttagatctgaaaacagttgcgctacatgcccgtaatgcagaatataaccccaagcgttttgctgctgtcatcatgcgtattagagagccaaaaactacagctttaatttttgcctcagggaaaatggttgttaccggtgcaaaaagtgaggatgactcaaagctggccagtagaaaatatgcaagaattatccaaaaaatcgggtttgctgctaaattcacagacttcaaaatacaaaatattgtcggttcgtgtgacgttaaattccctatacgtctagaagggttagcattcagtcatggtactttctcctcctatgagccagaattgtttcctggtttgatctatagaatggtgaagccgaaaattgtgttgttaatttttgtttcaggaaagattgttcttactggtgcaaagcaaagggaagaaatttaccaagcttttgaagctatataccctgtgctaagtgaatttagaaaaatgtga

SEQ ID NO: 9 - protein, 240 aa, Saccharomyces cerevisiae
MADEERLKEFKEANKIVFDPNTRQVWENQNRDGTKPATTFQSEEDIKRAAPESEKDTSATSGIVPTLQNIVATVTLGCRLDLKTVALHARNAEYNPKRFAAVIMRIREPKTTALIFASGKMVVTGAKSEDDSKLASRKYARIIQKIGFAAKFTDFKIQNIVGSCDVKFPIRLEGLAFSHGTFSSYEPELFPGLIYRMVKPKIVLLIFVSGKIVLTGAKQREEIYQAFEAIYPVLSEFRKM